European Patent Application EP 4 144 849 A1, published March 8, 2023. Title: Method for obtaining wheat with increased resistance to powdery mildew. Applicant: Suzhou Qi Biodesign biotechnology Company Limited. The sequence listing filed with the application follows.

SEQUENCE LISTING (12 sequences)

SEQ ID NO: 1 - DNA, 1605 bp, Triticum aestivum
atggcaaaggacgacgggtaccccccggcgcggacgctgccggagacgccgtcctgggcggtggcgctggtcttcgccgtcatgatcatcgtctccgtcctcctggagcacgcgctccacaagctcggccattggttccacaagcggcacaagaacgcgctggcggaggcgctggagaagatgaaggcggagctgatgctggtgggattcatctcgctgctgctcgccgtcacgcaggacccaatctccgggatatgcatctcccagaaggccgccagcatcatgcgcccctgcaaggtggaacccggttccgtcaagagcaagtacaaggactactactgcgccaaagagggcaaggtggcgctcatgtccacgggcagcctgcaccagctccacatattcatcttcgtgctagccgtcttccatgtcacctacagcgtcatcatcatggctctaagccgtctcaagatgagaacatggaagaaatgggagacagagaccgcctccttggaataccagttcgcaaatgatcctgcgcggttccgcttcacgcaccagacgtcgttcgtgaagcggcacctgggcctgtccagcacccccggcgtcagatgggtggtggccttcttcaggcagttcttcaggtcggtcaccaaggtggactacctcaccttgagggcaggcttcatcaacgcgcacttgtcgcagaacagcaagttcgacttccacaagtacatcaagaggtccatggaggacgacttcaaagtcgtcgttggcatcagcctcccgctgtgggctgtggcgatcctcaccctcttccttgatatcgacgggatcggcacactcacctgggtttctttcatccctctcatcatcctcttgtgtgttggaaccaagctagagatgatcatcatggagatggccctggagatccaggaccggtcgagcgtcatcaagggggcacccgtggtcgagcccagcaacaagttcttctggttccaccgccccgactgggtcctcttcttcatacacctgacgctgttccagaacgcgtttcagatggcacatttcgtgtggacagtggccacgcccggcttgaaggactgcttccatatgaacatcgggctgagcatcatgaaggtcgtgctggggctggctctccagttcctgtgcagctacatcaccttccccctctacgcgctagtcacacagatgggatcaaacatgaagaggtccatcttcgacgagcagacagccaaggcgctgaccaactggcggaacacggccaaggagaagaagaaggtccgagacacggacatgctgatggcgcagatgatcggcgacgcaacacccagccgaggcacgtccccgatgcctagccggggctcatcgccggtgcacctgcttcagaagggcatgggacggtctgacgatccccagagcgcaccgacctcgccaaggaccatggaggaggctagggacatgtacccggttgtggtggcgcatcctgtacacagactaaatcctgctgacaggcggaggtcggtctcttcatcagccctcgatgccgacatccccagcgcagatttttccttcagccagggatga

SEQ ID NO: 2 - protein, 534 aa, Triticum aestivum
MAKDDGYPPARTLPETPSWAVALVFAVMIIVSVLLEHALHKLGHWFHKRHKNALAEALEKMKAELMLVGFISLLLAVTQDPISGICISQKAASIMRPCKVEPGSVKSKYKDYYCAKEGKVALMSTGSLHQLHIFIFVLAVFHVTYSVIIMALSRLKMRTWKKWETETASLEYQFANDPARFRFTHQTSFVKRHLGLSSTPGVRWVVAFFRQFFRSVTKVDYLTLRAGFINAHLSQNSKFDFHKYIKRSMEDDFKVVVGISLPLWAVAILTLFLDIDGIGTLTWVSFIPLIILLCVGTKLEMIIMEMALEIQDRSSVIKGAPVVEPSNKFFWFHRPDWVLFFIHLTLFQNAFQMAHFVWTVATPGLKDCFHMNIGLSIMKVVLGLALQFLCSYITFPLYALVTQMGSNMKRSIFDEQTAKALTNWRNTAKEKKKVRDTDMLMAQMIGDATPSRGTSPMPSRGSSPVHLLQKGMGRSDDPQSAPTSPRTMEEARDMYPVVVAHPVHRLNPADRRRSVSSSALDADIPSADFSFSQG

SEQ ID NO: 3 - DNA, 1605 bp, Triticum aestivum
atggcggacgacgacgagtaccccccagcgaggacgctgccggagacgccgtcctgggcggtggccctcgtcttcgccgtcatgatcatcgtgtccgtcctcctggagcacgcgctccataagctcggccattggttccacaagcggcacaagaacgcgctggcggaggcgctggagaagatcaaggcggagctcatgctggtgggcttcatctcgctgctgctcgccgtgacgcaggaccccatctccgggatatgcatctccgagaaggccgccagcatcatgcggccctgcaagctgccccctggctccgtcaagagcaagtacaaagactactactgcgccaaacagggcaaggtgtcgctcatgtccacgggcagcttgcaccagctgcacatattcatcttcgtgctcgccgtcttccatgtcacctacagcgtcatcatcatggctctaagccgtctcaaaatgagaacctggaagaaatgggagacagagaccgcctccctggaataccagttcgcaaatgatcctgcgcggttccgcttcacgcaccagacgtcgttcgtgaagcggcacctgggcctctccagcacccccggcgtcagatgggtggtggccttcttcaggcagttcttcaggtcggtcaccaaggtggactacctcaccttgagggcaggcttcatcaacgcgcatttgtcgcataacagcaagttcgacttccacaagtacatcaagaggtccatggaggacgacttcaaagtcgtcgttggcatcagcctcccgctgtggtgtgtggcgatcctcaccctcttccttgacattgacgggatcggcacgctcacctggatttctttcatccctctcgtcatcctcttgtgtgttggaaccaagctggagatgatcatcatggagatggccctggagatccaggaccgggcgagcgtcatcaagggggcgcccgtggttgagcccagcaacaagttcttctggttccaccgccccgactgggtcctcttcttcatacacctgacgctattccagaacgcgtttcagatggcacatttcgtgtggacagtggccacgcccggcttgaagaaatgcttccatatgcacatcgggctgagcatcatgaaggtcgtgctggggctggctcttcagttcctctgcagctatatcaccttcccgctctacgcgctcgtcacacagatgggatcaaacatgaagaggtccatcttcgacgagcagacggccaaggcgctgacaaactggcggaacacggccaaggagaagaagaaggtccgagacacggacatgctgatggcgcagatgatcggcgacgcgacgcccagccgaggggcgtcgcccatgcctagccggggctcgtcgccagtgcacctgcttcacaagggcatgggacggtccgacgatccccagagcacgccaacctcgccaagggccatggaggaggctagggacatgtacccggttgtggtggcgcatccagtgcacagactaaatcctgctgacaggagaaggtcggtctcgtcgtcggcactcgatgtcgacattcccagcgcagatttttccttcagccagggatga

SEQ ID NO: 4 - protein, 534 aa, Triticum aestivum
MADDDEYPPARTLPETPSWAVALVFAVMIIVSVLLEHALHKLGHWFHKRHKNALAEALEKIKAELMLVGFISLLLAVTQDPISGICISEKAASIMRPCKLPPGSVKSKYKDYYCAKQGKVSLMSTGSLHQLHIFIFVLAVFHVTYSVIIMALSRLKMRTWKKWETETASLEYQFANDPARFRFTHQTSFVKRHLGLSSTPGVRWVVAFFRQFFRSVTKVDYLTLRAGFINAHLSHNSKFDFHKYIKRSMEDDFKVVVGISLPLWCVAILTLFLDIDGIGTLTWISFIPLVILLCVGTKLEMIIMEMALEIQDRASVIKGAPVVEPSNKFFWFHRPDWVLFFIHLTLFQNAFQMAHFVWTVATPGLKKCFHMHIGLSIMKVVLGLALQFLCSYITFPLYALVTQMGSNMKRSIFDEQTAKALTNWRNTAKEKKKVRDTDMLMAQMIGDATPSRGASPMPSRGSSPVHLLHKGMGRSDDPQSTPTSPRAMEEARDMYPVVVAHPVHRLNPADRRRSVSSSALDVDIPSADFSFSQG

SEQ ID NO: 5 - DNA, 1605 bp, Triticum aestivum
atggcggaggactacgagtaccccccggcgcggacgctgccggagacgccgtcctgggcggtggcgctcgtcttcgccgtcatgatcatcgtgtccgtcctcctggagcacgcgctccacaagctcggccattggttccacaagcggcacaagaacgcgctggcggaggcgctggagaagatcaaagcggagctgatgctggtggggttcatctcgctgctgctcgccgtgacgcaggacccaatctccgggatatgcatctccgagaaggccgccagcatcatgcggccctgcagcctgccccctggttccgtcaagagcaagtacaaagactactactgcgccaaaaagggcaaggtgtcgctaatgtccacgggcagcttgcaccagctccacatattcatcttcgtgctcgccgtcttccatgtcacctacagcgtcatcatcatggctctaagccgtctcaaaatgaggacatggaagaaatgggagacagagaccgcctccttggaataccagttcgcaaatgatcctgcgcggttccgcttcacgcaccagacgtcgttcgtgaagcgtcacctgggcctctccagcacccccggcatcagatgggtggtggccttcttcaggcagttcttcaggtcggtcaccaaggtggactacctcaccctgagggcaggcttcatcaacgcgcatttgtcgcataacagcaagttcgacttccacaagtacatcaagaggtccatggaggacgacttcaaagtcgtcgttggcatcagcctcccgctgtggtgtgtggcgatcctcaccctcttccttgatattgacgggatcggcacgctcacctggatttctttcatccctctcgtcatcctcttgtgtgttggaaccaagctggagatgatcatcatggagatggccctggagatccaggaccgggcgagcgtcatcaagggggcgcccgtggttgagcccagcaacaagttcttctggttccaccgccccgactgggtcctcttcttcatacacctgacgctgttccagaatgcgtttcagatggcacatttcgtctggacagtggccacgcccggcttgaagaaatgcttccatatgcacatcggtctgagcatcatgaaggtcgtgctggggctggctcttcagttcctctgcagctatatcaccttccccctctacgcgctcgtcacacagatgggatcgaacatgaagaggtccatcttcgacgagcagacggccaaggcgctgaccaactggcggaacacggccaaggagaagaagaaggtccgagacacggacatgctgatggcgcagatgatcggcgacgcgacgcccagccgaggcacgtcgccgatgcctagccgggcttcgtcaccggtgcacctgcttcacaagggcatgggacggtccgacgatccccagagcgcgccgacctcgccaaggaccatggaggaggctagggacatgtacccggttgtggtggcgcatcccgtgcacagactaaatcctgctgacaggcggaggtcggtctcttcgtcggcactcgatgccgacatccccagcgcagatttttccttcagccagggatga

SEQ ID NO: 6 - protein, 534 aa, Triticum aestivum
MAEDYEYPPARTLPETPSWAVALVFAVMIIVSVLLEHALHKLGHWFHKRHKNALAEALEKIKAELMLVGFISLLLAVTQDPISGICISEKAASIMRPCSLPPGSVKSKYKDYYCAKKGKVSLMSTGSLHQLHIFIFVLAVFHVTYSVIIMALSRLKMRTWKKWETETASLEYQFANDPARFRFTHQTSFVKRHLGLSSTPGIRWVVAFFRQFFRSVTKVDYLTLRAGFINAHLSHNSKFDFHKYIKRSMEDDFKVVVGISLPLWCVAILTLFLDIDGIGTLTWISFIPLVILLCVGTKLEMIIMEMALEIQDRASVIKGAPVVEPSNKFFWFHRPDWVLFFIHLTLFQNAFQMAHFVWTVATPGLKKCFHMHIGLSIMKVVLGLALQFLCSYITFPLYALVTQMGSNMKRSIFDEQTAKALTNWRNTAKEKKKVRDTDMLMAQMIGDATPSRGTSPMPSRASSPVHLLHKGMGRSDDPQSAPTSPRTMEEARDMYPVVVAHPVHRLNPADRRRSVSSSALDADIPSADFSFSQG

SEQ ID NO: 7 - DNA, 2223 bp, Triticum aestivum
atggaagatttaacacggcctcttgtgagagagtcggaggctaatcttcatgcgaagctcgctccctccggctccggatctggactacgacaagcgtgtaagaagttgcgtgatttgacgaccgttgatcgcgcggttcttgtcgcgttcgtggcatccatcggcaacctgctccaaggctgggacaatgccagcattgcaggtgctatgttttacataaaggacgagtttaaactagatagcatgccaatgattgaggggtgtattatggctatggcactttttggggcaacaataatcacaacactatctggaatgctatctgataaatttggtcggtgggcgatgctacttacctcggcggtattgtcctttgttagtgcactattggtcatattttggtcccaacatgtgtatatgctgctattcgtgaggcttattcagggatttagtattggtttggcagttacacttgtgccattatatatagttgagactgcgcctcctgatatgagaggaaaattaagcacatttccccagttaagtggttcagctggtatgttcttatcttactgcatggtgttttggatgtccatgctgccaaaggttagttggcggatcatgcttgggatacaactgataccctcactaatatactcaattttaactatcttctatctacctgagactccgagttggcttgtgagccaaggaagggtggatgaagccaagatggttttacaaaaactacgaagaaaggaagatgtctcaggtgaaatggcaagtcttttggagggcacacaagttggtgacactccgtctattgaggagtacctaattagcactaacgaaagtatgttaagggaaaaggtgattggcaatgatgaaataataaaattatatggacttccagaagatttgcattgtgttgcctatccattgaagagaacaaacacagaagaaagtgccattggtcattctgtgagtcgtggagcatcgttctatgacccagttgtcaacattattgggagtatgcacgggctccctgaggttgcccacggcatattcaatgaattagaacaacaaggtccaattgaaggggatgaagagaatcaggaagagaccaaagagcatgagctagaacacaaccgagatgatacctatgatagcgagcatgattatcttattcaacccaaacctacgaatataaatgattttgtgatatgtcgcaaaagcggccatattggtggaggttggcaattggcttggaaaatgtcatcaggatatcatttggatgggcaaatggaaggtggcatggaacgagtatatttgcatgaaggaggtgtaccaagttctgaaaatctactggatgctccaatagacgggaatttcattcaagcgactgctttggtcaacaaatcggtttttcacaagtctggacacaatattggtattcattcacctaataaagattatagaagtacaaaatggaaggatctgttagaacctggtgtaaaacgtgcattggtcgtgggtgttggaatacaagtacttcaacagtttgctggcatcaatggcattctttattacactcctcaaatacttgagcaagctggtgttggggttcttctctcaaagtttggcatcaactcttcttcagtgtcgattcttatgagcgctctcacaactttattgatgcttccttttatctgcatagccatgtggcttatggaccgctctggaagaagaaggatactacttgtgacaatacccatcttggtagtgtccctcgttgttttagtaaccgtcaacattgtgaatctgagtgctgaactacacgcactgctctcaacaatgagtgttggaatctatttctgcatatttgtcatgggttttggtccaataccaaatatattctgctcagagattttccccaacaaagttcgtgctatttgcttggccatatgtagcctagtcttttggatttgtgacatcattgtgacatatacccttcctgtattgttgaggtatataggtcttgcgggtgttttcggagtttatgccattgtttgtgtgttggcttttgttttcgtttgtctaaaggtcccggaaacaaagaatatacctattgaggtcatagcagagttctatgcacttggcgggtcaggtacccaaatcatccaagagaggcagaaagaaaattcagagaaattattagtgtga

SEQ ID NO: 8 - protein, 740 aa, Triticum aestivum
MEDLTRPLVRESEANLHAKLAPSGSGSGLRQACKKLRDLTTVDRAVLVAFVASIGNLLQGWDNASIAGAMFYIKDEFKLDSMPMIEGCIMAMALFGATIITTLSGMLSDKFGRWAMLLTSAVLSFVSALLVIFWSQHVYMLLFVRLIQGFSIGLAVTLVPLYIVETAPPDMRGKLSTFPQLSGSAGMFLSYCMVFWMSMLPKVSWRIMLGIQLIPSLIYSILTIFYLPETPSWLVSQGRVDEAKMVLQKLRRKEDVSGEMASLLEGTQVGDTPSIEEYLISTNESMLREKVIGNDEIIKLYGLPEDLHCVAYPLKRTNTEESAIGHSVSRGASFYDPVVNIIGSMHGLPEVAHGIFNELEQQGPIEGDEENQEETKEHELEHNRDDTYDSEHDYLIQPKPTNINDFVICRKSGHIGGGWQLAWKMSSGYHLDGQMEGGMERVYLHEGGVPSSENLLDAPIDGNFIQATALVNKSVFHKSGHNIGIHSPNKDYRSTKWKDLLEPGVKRALVVGVGIQVLQQFAGINGILYYTPQILEQAGVGVLLSKFGINSSSVSILMSALTTLLMLPFICIAMWLMDRSGRRRILLVTIPILVVSLVVLVTVNIVNLSAELHALLSTMSVGIYFCIFVMGFGPIPNIFCSEIFPNKVRAICLAICSLVFWICDIIVTYTLPVLLRYIGLAGVFGVYAIVCVLAFVFVCLKVPETKNIPIEVIAEFYALGGSGTQIIQERQKENSEKLLV

SEQ ID NO: 9 - DNA, 2226 bp, Triticum aestivum
atggaagatttatcacgccctcttgtgagagactcggaggctaatcttcatgccaagctcgctccctctggccacggatctggactactacaacaagcgtgtcagaagttgcgtgacttgacgaccgttgatcgcgcggtcctcgtcgcgttcgtggcatccatcggcaacctgctccaaggctgggacaatgcgagcattgcaggtgctatgctttacataaaggatgagtttaaactagatagcatgccaatgattgaggggtgcattatggctatggcactttttggggcaacaataatcacaacactatctggaatgctatctaataaatttggtaggtgggcgatgctacttacctcggcggtattgtcctttgttagtgcactattggtcatattttggtcccaacatgtgtatatgctgctattcgcgaggcttattcagggatttagtattggtttggcagttacacttgtgccattatatatagttgagaccgcacctcctgatatgagaggaaaattaagcacatttccccagttaagtggttcagttggtatgttcttatcttactgcatggtgttttggatgtccatgctgccaaaggttagttggcgggtcatgcttgggatacaactgataccctcactaatatactcaattttaacaatcttctatctacccgagactccgagttggcttgtgagccaaggaagggtggatgaagcaaagatggttttacaaaaactacgaagaaaggaagatgtctcaggtgaaatggcaagtcttttggagggcacacaagttggtgacactccgtctattgaggagtacctaattagcactaatgaaagtatgttaagggaaaaagtgattggcaatgatgaaataataaaattatatggacttccagaagatttgcattgtgttgcctatccattgaagagaacaaacacagaagaaagtgccattggtcattctgtgagtcatggagcatcgttctatgacccagttgtcaacattattgggagtatgcacgggctccccgaggttgcccacggcatattcaatgaattagaacaacaaggtccaattgaaggggacgaagagaatcaggaagagaccaaagagcatgagctagaacacaaccgagatggtacctatgatagcgagcatgcttatcttattcaacccaaacctacgaatataaatgattttgtggtatgtcgcaaaagcggccatattggtggaggttggcaattggcttggaaaatgtcatcaggatatcgtttagatgggcaaatggaaggtggcatggaacgagtatatttgcatgaaggaggtgtaccaagttctgaaaacctactggatgctccaatagatgggaatttcattcaagcgactgctttggtcaataaatcggtttttcataagtctggacacaatattggtattcattcacctaacaaagattatagaagtacaaaatggaaggatctgttagaacctggtgtaaaacgtgcattggtcgtgggtgttggaatacaagtgcttcaacagtttgctggcatcaatggcattctttattacactcctcaaatacttgagcaagctggtattggggttcttctctcaaagtttggcatcagctcttcttcagtgtcgattcttatgagcgctctcacaactttattgatgcttccttttatttgcatggccatgtggcttatggaccgctctggaagaagaaggatactacttgtgacaatacccatcttggtagtgtccctcattgttttggtaaccgtcaacattgtgaatctgagtgctgaactacacgcactgctctcaacaatgagtgttggaatctatttctgcatatttgtcatgggttttggtccaataccaaatatattctgctcggagattttccccaacaaagttcgtgctatttgcttggccatatgtagcctaatcttttggatttgtgacatcattgtgacatataccctccctgtattgttgaggtatataggtcttgcgggtgttttcggagtttatgccattgtttgtgtgctggcttttgttttcgtttgtctaaaggtcccggaaacaaagaatatacctattgaggtcatagaagagttctatgcacttggcgggtcagacacccaaatcatccaagagaggaagaaagaaaattcagagaaattattagtgtga

SEQ ID NO: 10 - protein, 741 aa, Triticum aestivum
MEDLSRPLVRDSEANLHAKLAPSGHGSGLLQQACQKLRDLTTVDRAVLVAFVASIGNLLQGWDNASIAGAMLYIKDEFKLDSMPMIEGCIMAMALFGATIITTLSGMLSNKFGRWAMLLTSAVLSFVSALLVIFWSQHVYMLLFARLIQGFSIGLAVTLVPLYIVETAPPDMRGKLSTFPQLSGSVGMFLSYCMVFWMSMLPKVSWRVMLGIQLIPSLIYSILTIFYLPETPSWLVSQGRVDEAKMVLQKLRRKEDVSGEMASLLEGTQVGDTPSIEEYLISTNESMLREKVIGNDEIIKLYGLPEDLHCVAYPLKRTNTEESAIGHSVSHGASFYDPVVNIIGSMHGLPEVAHGIFNELEQQGPIEGDEENQEETKEHELEHNRDGTYDSEHAYLIQPKPTNINDFVVCRKSGHIGGGWQLAWKMSSGYRLDGQMEGGMERVYLHEGGVPSSENLLDAPIDGNFIQATALVNKSVFHKSGHNIGIHSPNKDYRSTKWKDLLEPGVKRALVVGVGIQVLQQFAGINGILYYTPQILEQAGIGVLLSKFGISSSSVSILMSALTTLLMLPFICMAMWLMDRSGRRRILLVTIPILVVSLIVLVTVNIVNLSAELHALLSTMSVGIYFCIFVMGFGPIPNIFCSEIFPNKVRAICLAICSLIFWICDIIVTYTLPVLLRYIGLAGVFGVYAIVCVLAFVFVCLKVPETKNIPIEVIEEFYALGGSDTQIIQERKKENSEKLLV

SEQ ID NO: 11 - DNA, 2223 bp, Triticum aestivum
atggaagatttaacgcgtcctcttgtgagagattcggaggctaatcttcatgccaagctcgctccctccggctccggatctggactgcaacaagcgtgtaagaagttgcgtgatttgacgaccgttgatcgcgcggttcttgtcgcgttcgtggcatccatcggcaacctgctccaaggctgggacaatgcgagcattgcaggtgctatgttttacataaaggatgagtttaaactagatagcatgctaatgattgaggggtgtattatggccatggcactttttggggcaacaataatcacaacactatctggaatgctatctgataaatttggtaggtgggcgatgctacttacctcggcggtgttgtcctttgttagtgcagtattggtcatattttggtcccaacatgtgtatatgctgctattcgcgaggcttattcagggatttagcattggtttggcagttacacttgtgccattatatatagttgagaccgcgcctcctgatatgagaggaaaattaagcacatttccccagttaagtggttcagttggtatgttcttgtcttactgcatggtgttttggatgtccatgctgccaaaggttagttggcggatcatgcttgggatacaactgataccctcactaatatactcaattttaactatcttctatctacccgagactccgagttggcttgtgagccaaggaagggtggatgaagccaagatggttttacaaaaactacgaagaaaggaagatgtctcaggtgaaatggcaagtcttttggagggtacacaagttggtgatactccgtctattgaggagtacctaattagcactaatgaaagtatgttaagggaaaaagtgattggcaatgatgaaataataaaattatatggacttccggaagatttgcattgtgttgcctatccattgaagagaacaaacacagaagaaagtgccattggtcattctgtgagtcgtggagcatcgttctatgacccagttgtcaacattattgggagtatgcacgggctccctgaggttgcccacggcatattcaatgaattagaacaacaaggtccaattgaaggggacgaagagaatcaggaagagaccaaagagcatgagctagaacacaaccgagatgatacctatgatagcgagcatgattatcttattcaacccaaacctacgaatataaatgattttgttgtatgtcgcaaaagcggccatattggtggaggttggcaattggcttggaaaatgtcatcaggatatcatttggatgggcaaatggaaggtggcatggaacgggtatatttgcatgaaggaggtgtaccaagttctgaaaacctactagatgctccaatagacgggaatttcattcaagcgactgctttggtcaacaaatcggtttttcataagtctggacacaatattggtattcattcacctaataaagattatagaagtacaaaatggaaggatctgttagaacctggtgtaaaacgtgcattggtcgtgggtgttggaatacaagtacttcaacagtttgctggcatcaatggcattctttattacactccacaaatacttgagcaagctggtgttggggttcttctctcaaagtttggcatcaactcttcttcagtgtcgattcttatgagcgctctcacaactttattgatgcttccttttatttgcatagccatgtggcttatggaccgctctggaagaagaaggatactacttgtgacaatacccatcttggttgtgtccctcattgttttggtaacagtcaacattgtgaatctgagtgctgaactacacgcactgctctcaacaatgagtgttggaatctatttctgcatatttgtcatgggttttggtccaataccaaatatattctgctcggagattttccccaacaaagttcgtgctatttgcttggccatatgtagccttatcttttggatttgtgacatcattgtgacatataccctccctgtattgttgaggtatataggtcttgcgggtgtttttggagtttatgccattgtttgtgtgctggcttttgttttcgtttgtttaaaggtcccggaaacaaagaatatacctattgaggtcatagcagagttctatgcacttggcgggtcaggtacccaaatcatccaagagaggcagaaagaaaattcagagaaattattagcgtga

SEQ ID NO: 12 - protein, 740 aa, Triticum aestivum
MEDLTRPLVRDSEANLHAKLAPSGSGSGLQQACKKLRDLTTVDRAVLVAFVASIGNLLQGWDNASIAGAMFYIKDEFKLDSMLMIEGCIMAMALFGATIITTLSGMLSDKFGRWAMLLTSAVLSFVSAVLVIFWSQHVYMLLFARLIQGFSIGLAVTLVPLYIVETAPPDMRGKLSTFPQLSGSVGMFLSYCMVFWMSMLPKVSWRIMLGIQLIPSLIYSILTIFYLPETPSWLVSQGRVDEAKMVLQKLRRKEDVSGEMASLLEGTQVGDTPSIEEYLISTNESMLREKVIGNDEIIKLYGLPEDLHCVAYPLKRTNTEESAIGHSVSRGASFYDPVVNIIGSMHGLPEVAHGIFNELEQQGPIEGDEENQEETKEHELEHNRDDTYDSEHDYLIQPKPTNINDFVVCRKSGHIGGGWQLAWKMSSGYHLDGQMEGGMERVYLHEGGVPSSENLLDAPIDGNFIQATALVNKSVFHKSGHNIGIHSPNKDYRSTKWKDLLEPGVKRALVVGVGIQVLQQFAGINGILYYTPQILEQAGVGVLLSKFGINSSSVSILMSALTTLLMLPFICIAMWLMDRSGRRRILLVTIPILVVSLIVLVTVNIVNLSAELHALLSTMSVGIYFCIFVMGFGPIPNIFCSEIFPNKVRAICLAICSLIFWICDIIVTYTLPVLLRYIGLAGVFGVYAIVCVLAFVFVCLKVPETKNIPIEVIAEFYALGGSGTQIIQERQKENSEKLLA